European Patent Specification EP 4 158 055 B1, published March 27, 2024. Title: OLIGONUCLEOTIDES AND BEADS FOR 5 PRIME GENE EXPRESSION ASSAY. Applicant: BECTON, DICKINSON AND COMPANY Lazaruk, Katherine. The sequence listing filed with the application follows.

SEQUENCE LISTING (2 sequences)

SEQ ID NO: 1 - DNA, 107 bp, Artificial Sequence
  Bead-associated oligonucleotide comprising polyT capture sequence
  misc_feature (82)..(89): n is a, c, g, or t
tctctctctacacgacgctcttccgatctatcacgttaactggcctgcgacgatgtttaggtagcggtgacattaggcatannnnnnnntttttttttttttttttt

SEQ ID NO: 2 - DNA, 102 bp, Artificial Sequence
  Bead-associated oligonucleotide comprising specific capture sequence
  misc_feature (79)..(86): n is a, c, g, or t
tctctctcggaaccttggaattccggatcacgttaactggcctgcgacgatgtttaggtagcggtgacattaggcatannnnnnnnacgtacgtacgtacgt